European Patent Application EP 4 435 012 A1, published September 25, 2024. Title: BCMA-TARGETING CHIMERIC ANTIGEN RECEPTOR AND USE THEREOF. Applicant: JUVENTAS CELL THERAPY LTD. The sequence listing filed with the application follows.

SEQUENCE LISTING (41 sequences)

SEQ ID NO: 1 - protein, 8 aa, synthetic construct
GFSLSTYH

SEQ ID NO: 2 - protein, 7 aa, synthetic construct
ISSSGST

SEQ ID NO: 3 - protein, 10 aa, synthetic construct
ARDLDYVIDL

SEQ ID NO: 4 - protein, 7 aa, synthetic construct
PSVYNNY

SEQ ID NO: 5 - skipped

SEQ ID NO: 6 - protein, 11 aa, synthetic construct
AGTYVSGDRRA

SEQ ID NO: 7 - protein, 116 aa, synthetic construct
EVQLVESGGGLVQPGGSLRLSCTASGFSLSTYHMTWVRQAPGKGLEWIGVISSSGSTYYASWAKGRFTISRDNSKNTVYLQMNSLRAEDTAVYFCARDLDYVIDLWGPGTLVTVSS

SEQ ID NO: 8 - protein, 110 aa, synthetic construct
EIVMTQSPSTLSASVGDRVIINCQSSPSVYNNYLSWYQQKPGKAPKLLIYETSTLASGVPSRFSGSGSGAEFTLTISSLQPDDFATYYCAGTYVSGDRRAFGQGTKLTVL

SEQ ID NO: 9 - protein, 114 aa, synthetic construct
QSVEESGGRLVTPGTPLTLTCTASGFSLSTYHMTWVRQAPGKGLEWIGVISSSGSTYYASWAKGRFTISKTSSTTVDLKMTSLTTEDTATYFCARDLDYVIDLWGQGTLVTVSS

SEQ ID NO: 10 - protein, 110 aa, synthetic construct
AQVLTQTPSSVSSAVGGTVTINCQSSPSVYNNYLSWFQQKPGQPPKLLIYETSTLPSGVPSRFSASGSGTQFTLTISGVQCDDAATYYCAGTYVSGDRRAFGGGTEVVVK

SEQ ID NO: 11 - protein, 241 aa, synthetic construct
EIVMTQSPSTLSASVGDRVIINCQSSPSVYNNYLSWYQQKPGKAPKLLIYETSTLASGVPSRFSGSGSGAEFTLTISSLQPDDFATYYCAGTYVSGDRRAFGQGTKLTVLGGGGSGGGGSGGGGSEVQLVESGGGLVQPGGSLRLSCTASGFSLSTYHMTWVRQAPGKGLEWIGVISSSGSTYYASWAKGRFTISRDNSKNTVYLQMNSLRAEDTAVYFCARDLDYVIDLWGPGTLVTVSS

SEQ ID NO: 12 - protein, 239 aa, synthetic construct
AQVLTQTPSSVSSAVGGTVTINCQSSPSVYNNYLSWFQQKPGQPPKLLIYETSTLPSGVPSRFSASGSGTQFTLTISGVQCDDAATYYCAGTYVSGDRRAFGGGTEVVVKGGGGSGGGGSGGGGSQSVEESGGRLVTPGTPLTLTCTASGFSLSTYHMTWVRQAPGKGLEWIGVISSSGSTYYASWAKGRFTISKTSSTTVDLKMTSLTTEDTATYFCARDLDYVIDLWGQGTLVTVSS

SEQ ID NO: 13 - protein, 45 aa, synthetic construct
TTTPAPRPPTPAPTIASQPLSLRPEACRPAAGGAVHTRGLDFACD

SEQ ID NO: 14 - protein, 24 aa, synthetic construct
IYIWAPLAGTCGVLLLSLVITLYC

SEQ ID NO: 15 - protein, 112 aa, synthetic construct
RVKFSRSADAPAYQQGQNQLYNELNLGRREEYDVLDKRRGRDPEMGGKPRRKNPQEGLYNELQKDKMAEAYSEIGMKGERRRGKGHDGLYQGLSTATKDTYDALHMQALPPR

SEQ ID NO: 16 - protein, 42 aa, synthetic construct
KRGRKKLLYIFKQPFMRPVQTTQEEDGCSCRFPEEEEGGCEL

SEQ ID NO: 17 - protein, 21 aa, synthetic construct
MALPVTALLLPLALLLHAARP

SEQ ID NO: 18 - DNA, 723 bp, synthetic construct
  source 1..723: mol_type = other DNA
gagatcgtgatgacccagtccccaagtacactgagcgcctccgtgggcgaccgcgtgatcataaactgtcaaagctcaccctctgtttacaacaattacctgtcttggtatcaacagaagcccggtaaggcccccaaactgctcatttacgagacatccaccctggcatccggggtgccaagccgcttctccgggagtgggtctggcgccgagttcaccctgaccatatcttccctgcagcccgacgacttcgcaacgtactattgcgccggaacctatgtaagtggggatagacgcgccttcgggcagggcacgaagttgaccgtgctgggcggagggggctcaggaggtggcggtagcggaggaggcggctcagaagtgcagctggtggagtccggcggtggactggtgcaaccgggaggctcactcagattgtcatgcaccgcctctggctttagtctctccacctatcatatgacttgggtgaggcaggcacccggcaagggcctggaatggatcggcgtgatctcttccagcggtagcacctattacgcctcttgggcgaagggcaggtttaccatcagccgcgacaacagcaagaataccgtttacctgcagatgaatagcctgagggccgaagacacggcggtctatttctgtgcacgggaccttgactacgttattgacctgtggggccctgggaccctcgtaactgtgagcagc

SEQ ID NO: 19 - protein, 250 aa, synthetic construct
EIVMTQSPSTLSASVGDRVIITCQASENIYRNLAWYQQKPGKAPKLLIYAASLLASGVPSRFSGSGSGAEFTLTISSLQPDDFATYYCQNAFYSSSADNPFGQGTKLTVLGGGGSGGGGSGGGGSEVQLVESGGGLVQPGGSLRLSCTASGFSLSSYAMSWVRQAPGKGLEWIGMISSSGSTHYASWAKGRFTISRDTSKNTVYLQMNSLRAEDTAVYYCARDFYVYSSGTYLEYGMDLWGQGTLVTVSS

SEQ ID NO: 20 - protein, 252 aa, synthetic construct
EIVMTQSPSTLSASVGDRVIINCQSSPSVYNKNWLSWYQQKPGKAPKLLIYKASTLASGVPSRFSGSGSGAEFTLTISSLQPDDFATYYCAGGYNSDSERGTFGQGTKLTVLGGGGSGGGGSGGGGSEVQLVESGGGLVQPGGSLRLSCTASGFSLSSSYWICWVRQAPGKGLEWIGCVYVGSSDFTYYATWAKGRFTISRDNSKNTVYLQMNSLRAEDTAVYFCARPYPDWNIDSFRWDLWGPGTLVTVSS

SEQ ID NO: 21 - protein, 248 aa, synthetic construct
EIVMTQSPSTLSASVGDRVIINCQASQSVFSNNYLAWYQQKPGKAPKLLIYRASNLASGVPSRFSGSGSGAEFTLTISSLQPDDFATYYCQPTYLSGDWYVAFGQGTKLTVLGGGGSGGGGSGGGGSEVQLVESGGGLVQPGGSLRLSCTASGFSLNYYGMGWVRQAPGKGLEWIGIIAGDRDTYYATWAKGRFTISRDNSKNTVYLQMNSLRAEDTAVYFCARGSYSSTWDGAFDLWGPGTLVTVSS

SEQ ID NO: 22 - protein, 246 aa, synthetic construct
EIVMTQSPSTLSASVGDRVIINCQASQSIDSWLSWYQQKPGKAPKLLIYLASTLASGVPSRFSGSGSGAEFTLTISSLQPDDFATYYCQSNDESSIYGAAFGQGTKLTVLGGGGSGGGGSGGGGSEVQLVESGGGLVQPGGSLRLSCTASGFSLSIYDMIWVRQAPGKGLEWIGIIIYGGSASYANWAKGRFTISRDNSKNTVYLQMNSLRAEDTAVYFCARGASSYSYSYGFSLWGPGTLVTVSS

SEQ ID NO: 23 - DNA, 750 bp, synthetic construct
  source 1..750: mol_type = other DNA
gagatcgtgatgacccagtccccaagtacactgagcgcctccgtgggcgaccgcgtgatcataacctgtcaagcctctgagaatatctataggaacctggcctggtatcaacagaagcccggtaaggcccccaaactgctcatttacgccgccagcctgctggcatccggggtgccaagccgcttctccgggagtgggtctggcgccgagttcaccctgaccatatcttccctgcagcccgacgacttcgcaacgtactattgccagaacgccttctacagctctagcgcggacaaccccttcgggcagggcacgaagttgaccgtgctgggcggagggggctcaggaggtggcggtagcggaggaggcggctcagaagtgcagctggtggagtccggcggtggactggtgcaaccgggaggctcactcagattgtcatgcaccgcctctggctttagtttgtccagctatgcgatgagctgggtgaggcaggcacccggcaagggcctggaatggatcggcatgatcagctcctcaggttcaacccattacgcaagttgggcgaagggcaggtttaccatcagccgcgacaccagcaagaataccgtttacctgcagatgaatagcctgagggccgaagacacggcggtctattactgtgcacgggacttctatgtgtacagttccgggacgtacctcgagtatggcatggacctgtggggccaggggaccctcgtaactgtgagcagc

SEQ ID NO: 24 - DNA, 756 bp, synthetic construct
  source 1..756: mol_type = other DNA
gagatcgtgatgacccagtccccaagtacactgagcgcctccgtgggcgaccgcgtgatcataaactgtcagagctctccctccgtatataataagaactggttgagttggtatcaacagaagcccggtaaggcccccaaactgctcatttacaaagcctctactctggcatccggggtgccaagccgcttctccgggagtgggtctggcgccgagttcaccctgaccatatcttccctgcagcccgacgacttcgcaacgtactattgcgctggtggctataatagcgatagcgagcgcggtaccttcgggcagggcacgaagttgaccgtgctgggcggagggggctcaggaggtggcggtagcggaggaggcggctcagaagtgcagctggtggagtccggcggtggactggtgcaaccgggaggctcactcagattgtcatgcaccgcctctggctttagtctgagcagttcctactggatttgctgggtgaggcaggcacccggcaagggcctggaatggatcggctgtgtgtacgttgggtcatccgactttacatattacgcgacatgggcgaagggcaggtttaccatcagccgcgacaacagcaagaataccgtttacctgcagatgaatagcctgagggccgaagacacggcggtctatttctgtgcacggccctatcccgactggaatattgatagttttagatgggatctgtggggccctgggaccctcgtaactgtgagcagc

SEQ ID NO: 25 - DNA, 744 bp, synthetic construct
  source 1..744: mol_type = other DNA
gagatcgtgatgacccagtccccaagtacactgagcgcctccgtgggcgaccgcgtgatcataaactgtcaggctagtcagagcgtctttagcaataactacttggcctggtatcaacagaagcccggtaaggcccccaaactgctcatttacagagcctctaatctggcatccggggtgccaagccgcttctccgggagtgggtctggcgccgagttcaccctgaccatatcttccctgcagcccgacgacttcgcaacgtactattgccaacccacgtacctctccggggactggtatgtggcattcgggcagggcacgaagttgaccgtgctgggcggagggggctcaggaggtggcggtagcggaggaggcggctcagaagtgcagctggtggagtccggcggtggactggtgcaaccgggaggctcactcagattgtcatgcaccgcctctggctttagtctcaactactatggtatgggctgggtgaggcaggcacccggcaagggcctggaatggatcggcatcattgctggtgaccgggacacatactatgctacttgggcgaagggcaggtttaccatcagccgcgacaacagcaagaataccgtttacctgcagatgaatagcctgagggccgaagacacggcggtctatttctgtgcacggggttcatatagcagtacatgggatggtgcatttgacctgtggggccctgggaccctcgtaactgtgagcagc

SEQ ID NO: 26 - DNA, 738 bp, synthetic construct
  source 1..738: mol_type = other DNA
gagatcgtgatgacccagtccccaagtacactgagcgcctccgtgggcgaccgcgtgatcataaactgtcaggcctcccagtctatcgacagctggttgtcatggtatcaacagaagcccggtaaggcccccaaactgctcatttacctggcatccacactggcatccggggtgccaagccgcttctccgggagtgggtctggcgccgagttcaccctgaccatatcttccctgcagcccgacgacttcgcaacgtactattgccaaagtaacgatgagagtagcatctacggtgccgccttcgggcagggcacgaagttgaccgtgctgggcggagggggctcaggaggtggcggtagcggaggaggcggctcagaagtgcagctggtggagtccggcggtggactggtgcaaccgggaggctcactcagattgtcatgcaccgcctctggctttagtctttcaatttacgacatgatatgggtgaggcaggcacccggcaagggcctggaatggatcggcattattatttacgggggcagtgccagctacgcgaattgggcgaagggcaggtttaccatcagccgcgacaacagcaagaataccgtttacctgcagatgaatagcctgagggccgaagacacggcggtctatttctgtgcacggggtgcatcatcatacagttactcttatggcttctccctgtggggccctgggaccctcgtaactgtgagcagc

SEQ ID NO: 27 - protein, 494 aa, synthetic construct
MALPVTALLLPLALLLHAARPEIVMTQSPSTLSASVGDRVIITCQASENIYRNLAWYQQKPGKAPKLLIYAASLLASGVPSRFSGSGSGAEFTLTISSLQPDDFATYYCQNAFYSSSADNPFGQGTKLTVLGGGGSGGGGSGGGGSEVQLVESGGGLVQPGGSLRLSCTASGFSLSSYAMSWVRQAPGKGLEWIGMISSSGSTHYASWAKGRFTISRDTSKNTVYLQMNSLRAEDTAVYYCARDFYVYSSGTYLEYGMDLWGQGTLVTVSSTTTPAPRPPTPAPTIASQPLSLRPEACRPAAGGAVHTRGLDFACDIYIWAPLAGTCGVLLLSLVITLYCKRGRKKLLYIFKQPFMRPVQTTQEEDGCSCRFPEEEEGGCELRVKFSRSADAPAYQQGQNQLYNELNLGRREEYDVLDKRRGRDPEMGGKPRRKNPQEGLYNELQKDKMAEAYSEIGMKGERRRGKGHDGLYQGLSTATKDTYDALHMQALPPR

SEQ ID NO: 28 - protein, 485 aa, synthetic construct
MALPVTALLLPLALLLHAARPEIVMTQSPSTLSASVGDRVIINCQSSPSVYNNYLSWYQQKPGKAPKLLIYETSTLASGVPSRFSGSGSGAEFTLTISSLQPDDFATYYCAGTYVSGDRRAFGQGTKLTVLGGGGSGGGGSGGGGSEVQLVESGGGLVQPGGSLRLSCTASGFSLSTYHMTWVRQAPGKGLEWIGVISSSGSTYYASWAKGRFTISRDNSKNTVYLQMNSLRAEDTAVYFCARDLDYVIDLWGPGTLVTVSSTTTPAPRPPTPAPTIASQPLSLRPEACRPAAGGAVHTRGLDFACDIYIWAPLAGTCGVLLLSLVITLYCKRGRKKLLYIFKQPFMRPVQTTQEEDGCSCRFPEEEEGGCELRVKFSRSADAPAYQQGQNQLYNELNLGRREEYDVLDKRRGRDPEMGGKPRRKNPQEGLYNELQKDKMAEAYSEIGMKGERRRGKGHDGLYQGLSTATKDTYDALHMQALPPR

SEQ ID NO: 29 - protein, 496 aa, synthetic construct
MALPVTALLLPLALLLHAARPEIVMTQSPSTLSASVGDRVIINCQSSPSVYNKNWLSWYQQKPGKAPKLLIYKASTLASGVPSRFSGSGSGAEFTLTISSLQPDDFATYYCAGGYNSDSERGTFGQGTKLTVLGGGGSGGGGSGGGGSEVQLVESGGGLVQPGGSLRLSCTASGFSLSSSYWICWVRQAPGKGLEWIGCVYVGSSDFTYYATWAKGRFTISRDNSKNTVYLQMNSLRAEDTAVYFCARPYPDWNIDSFRWDLWGPGTLVTVSSTTTPAPRPPTPAPTIASQPLSLRPEACRPAAGGAVHTRGLDFACDIYIWAPLAGTCGVLLLSLVITLYCKRGRKKLLYIFKQPFMRPVQTTQEEDGCSCRFPEEEEGGCELRVKFSRSADAPAYQQGQNQLYNELNLGRREEYDVLDKRRGRDPEMGGKPRRKNPQEGLYNELQKDKMAEAYSEIGMKGERRRGKGHDGLYQGLSTATKDTYDALHMQALPPR

SEQ ID NO: 30 - protein, 492 aa, synthetic construct
MALPVTALLLPLALLLHAARPEIVMTQSPSTLSASVGDRVIINCQASQSVFSNNYLAWYQQKPGKAPKLLIYRASNLASGVPSRFSGSGSGAEFTLTISSLQPDDFATYYCQPTYLSGDWYVAFGQGTKLTVLGGGGSGGGGSGGGGSEVQLVESGGGLVQPGGSLRLSCTASGFSLNYYGMGWVRQAPGKGLEWIGIIAGDRDTYYATWAKGRFTISRDNSKNTVYLQMNSLRAEDTAVYFCARGSYSSTWDGAFDLWGPGTLVTVSSTTTPAPRPPTPAPTIASQPLSLRPEACRPAAGGAVHTRGLDFACDIYIWAPLAGTCGVLLLSLVITLYCKRGRKKLLYIFKQPFMRPVQTTQEEDGCSCRFPEEEEGGCELRVKFSRSADAPAYQQGQNQLYNELNLGRREEYDVLDKRRGRDPEMGGKPRRKNPQEGLYNELQKDKMAEAYSEIGMKGERRRGKGHDGLYQGLSTATKDTYDALHMQALPPR

SEQ ID NO: 31 - protein, 490 aa, synthetic construct
MALPVTALLLPLALLLHAARPEIVMTQSPSTLSASVGDRVIINCQASQSIDSWLSWYQQKPGKAPKLLIYLASTLASGVPSRFSGSGSGAEFTLTISSLQPDDFATYYCQSNDESSIYGAAFGQGTKLTVLGGGGSGGGGSGGGGSEVQLVESGGGLVQPGGSLRLSCTASGFSLSIYDMIWVRQAPGKGLEWIGIIIYGGSASYANWAKGRFTISRDNSKNTVYLQMNSLRAEDTAVYFCARGASSYSYSYGFSLWGPGTLVTVSSTTTPAPRPPTPAPTIASQPLSLRPEACRPAAGGAVHTRGLDFACDIYIWAPLAGTCGVLLLSLVITLYCKRGRKKLLYIFKQPFMRPVQTTQEEDGCSCRFPEEEEGGCELRVKFSRSADAPAYQQGQNQLYNELNLGRREEYDVLDKRRGRDPEMGGKPRRKNPQEGLYNELQKDKMAEAYSEIGMKGERRRGKGHDGLYQGLSTATKDTYDALHMQALPPR

SEQ ID NO: 32 - DNA, 1485 bp, synthetic construct
  source 1..1485: mol_type = other DNA
atggccttaccagtgaccgccttgctcctgccgctggccttgctgctccacgccgccaggccggagatcgtgatgacccagtccccaagtacactgagcgcctccgtgggcgaccgcgtgatcataacctgtcaagcctctgagaatatctataggaacctggcctggtatcaacagaagcccggtaaggcccccaaactgctcatttacgccgccagcctgctggcatccggggtgccaagccgcttctccgggagtgggtctggcgccgagttcaccctgaccatatcttccctgcagcccgacgacttcgcaacgtactattgccagaacgccttctacagctctagcgcggacaaccccttcgggcagggcacgaagttgaccgtgctgggcggagggggctcaggaggtggcggtagcggaggaggcggctcagaagtgcagctggtggagtccggcggtggactggtgcaaccgggaggctcactcagattgtcatgcaccgcctctggctttagtttgtccagctatgcgatgagctgggtgaggcaggcacccggcaagggcctggaatggatcggcatgatcagctcctcaggttcaacccattacgcaagttgggcgaagggcaggtttaccatcagccgcgacaccagcaagaataccgtttacctgcagatgaatagcctgagggccgaagacacggcggtctattactgtgcacgggacttctatgtgtacagttccgggacgtacctcgagtatggcatggacctgtggggccaggggaccctcgtaactgtgagcagcaccacgacgccagcgccgcgaccaccaacaccggcgcccaccatcgcgtcgcagcccctgtccctgcgcccagaggcgtgccggccagcggcggggggcgcagtgcacacgagggggctggacttcgcctgtgatatctacatctgggcgcccttggccgggacttgtggggtccttctcctgtcactggttatcaccctttactgcaaacggggcagaaagaaactcctgtatatattcaaacaaccatttatgagaccagtacaaactactcaagaggaagatggctgtagctgccgatttccagaagaagaagaaggaggatgtgaactgagagtgaagttcagcaggagcgcagacgcccccgcgtaccagcagggccagaaccagctctataacgagctcaatctaggacgaagagaggagtacgatgttttggacaagagacgtggccgggaccctgagatggggggaaagccgagaaggaagaaccctcaggaaggcctgtacaatgaactgcagaaagataagatggcggaggcctacagtgagattgggatgaaaggcgagcgccggaggggcaaggggcacgatggcctttaccagggtctcagtacagccaccaaggacacctacgacgcccttcacatgcaggccctgccccctcgctaa

SEQ ID NO: 33 - DNA, 1458 bp, synthetic construct
  source 1..1458: mol_type = other DNA
atggccttaccagtgaccgccttgctcctgccgctggccttgctgctccacgccgccaggccggagatcgtgatgacccagtccccaagtacactgagcgcctccgtgggcgaccgcgtgatcataaactgtcaaagctcaccctctgtttacaacaattacctgtcttggtatcaacagaagcccggtaaggcccccaaactgctcatttacgagacatccaccctggcatccggggtgccaagccgcttctccgggagtgggtctggcgccgagttcaccctgaccatatcttccctgcagcccgacgacttcgcaacgtactattgcgccggaacctatgtaagtggggatagacgcgccttcgggcagggcacgaagttgaccgtgctgggcggagggggctcaggaggtggcggtagcggaggaggcggctcagaagtgcagctggtggagtccggcggtggactggtgcaaccgggaggctcactcagattgtcatgcaccgcctctggctttagtctctccacctatcatatgacttgggtgaggcaggcacccggcaagggcctggaatggatcggcgtgatctcttccagcggtagcacctattacgcctcttgggcgaagggcaggtttaccatcagccgcgacaacagcaagaataccgtttacctgcagatgaatagcctgagggccgaagacacggcggtctatttctgtgcacgggaccttgactacgttattgacctgtggggccctgggaccctcgtaactgtgagcagcaccacgacgccagcgccgcgaccaccaacaccggcgcccaccatcgcgtcgcagcccctgtccctgcgcccagaggcgtgccggccagcggcggggggcgcagtgcacacgagggggctggacttcgcctgtgatatctacatctgggcgcccttggccgggacttgtggggtccttctcctgtcactggttatcaccctttactgcaaacggggcagaaagaaactcctgtatatattcaaacaaccatttatgagaccagtacaaactactcaagaggaagatggctgtagctgccgatttccagaagaagaagaaggaggatgtgaactgagagtgaagttcagcaggagcgcagacgcccccgcgtaccagcagggccagaaccagctctataacgagctcaatctaggacgaagagaggagtacgatgttttggacaagagacgtggccgggaccctgagatggggggaaagccgagaaggaagaaccctcaggaaggcctgtacaatgaactgcagaaagataagatggcggaggcctacagtgagattgggatgaaaggcgagcgccggaggggcaaggggcacgatggcctttaccagggtctcagtacagccaccaaggacacctacgacgcccttcacatgcaggccctgccccctcgctaa

SEQ ID NO: 34 - DNA, 1491 bp, synthetic construct
  source 1..1491: mol_type = other DNA
atggccttaccagtgaccgccttgctcctgccgctggccttgctgctccacgccgccaggccggagatcgtgatgacccagtccccaagtacactgagcgcctccgtgggcgaccgcgtgatcataaactgtcagagctctccctccgtatataataagaactggttgagttggtatcaacagaagcccggtaaggcccccaaactgctcatttacaaagcctctactctggcatccggggtgccaagccgcttctccgggagtgggtctggcgccgagttcaccctgaccatatcttccctgcagcccgacgacttcgcaacgtactattgcgctggtggctataatagcgatagcgagcgcggtaccttcgggcagggcacgaagttgaccgtgctgggcggagggggctcaggaggtggcggtagcggaggaggcggctcagaagtgcagctggtggagtccggcggtggactggtgcaaccgggaggctcactcagattgtcatgcaccgcctctggctttagtctgagcagttcctactggatttgctgggtgaggcaggcacccggcaagggcctggaatggatcggctgtgtgtacgttgggtcatccgactttacatattacgcgacatgggcgaagggcaggtttaccatcagccgcgacaacagcaagaataccgtttacctgcagatgaatagcctgagggccgaagacacggcggtctatttctgtgcacggccctatcccgactggaatattgatagttttagatgggatctgtggggccctgggaccctcgtaactgtgagcagcaccacgacgccagcgccgcgaccaccaacaccggcgcccaccatcgcgtcgcagcccctgtccctgcgcccagaggcgtgccggccagcggcggggggcgcagtgcacacgagggggctggacttcgcctgtgatatctacatctgggcgcccttggccgggacttgtggggtccttctcctgtcactggttatcaccctttactgcaaacggggcagaaagaaactcctgtatatattcaaacaaccatttatgagaccagtacaaactactcaagaggaagatggctgtagctgccgatttccagaagaagaagaaggaggatgtgaactgagagtgaagttcagcaggagcgcagacgcccccgcgtaccagcagggccagaaccagctctataacgagctcaatctaggacgaagagaggagtacgatgttttggacaagagacgtggccgggaccctgagatggggggaaagccgagaaggaagaaccctcaggaaggcctgtacaatgaactgcagaaagataagatggcggaggcctacagtgagattgggatgaaaggcgagcgccggaggggcaaggggcacgatggcctttaccagggtctcagtacagccaccaaggacacctacgacgcccttcacatgcaggccctgccccctcgctaa

SEQ ID NO: 35 - DNA, 1479 bp, synthetic construct
  source 1..1479: mol_type = other DNA
atggccttaccagtgaccgccttgctcctgccgctggccttgctgctccacgccgccaggccggagatcgtgatgacccagtccccaagtacactgagcgcctccgtgggcgaccgcgtgatcataaactgtcaggctagtcagagcgtctttagcaataactacttggcctggtatcaacagaagcccggtaaggcccccaaactgctcatttacagagcctctaatctggcatccggggtgccaagccgcttctccgggagtgggtctggcgccgagttcaccctgaccatatcttccctgcagcccgacgacttcgcaacgtactattgccaacccacgtacctctccggggactggtatgtggcattcgggcagggcacgaagttgaccgtgctgggcggagggggctcaggaggtggcggtagcggaggaggcggctcagaagtgcagctggtggagtccggcggtggactggtgcaaccgggaggctcactcagattgtcatgcaccgcctctggctttagtctcaactactatggtatgggctgggtgaggcaggcacccggcaagggcctggaatggatcggcatcattgctggtgaccgggacacatactatgctacttgggcgaagggcaggtttaccatcagccgcgacaacagcaagaataccgtttacctgcagatgaatagcctgagggccgaagacacggcggtctatttctgtgcacggggttcatatagcagtacatgggatggtgcatttgacctgtggggccctgggaccctcgtaactgtgagcagcaccacgacgccagcgccgcgaccaccaacaccggcgcccaccatcgcgtcgcagcccctgtccctgcgcccagaggcgtgccggccagcggcggggggcgcagtgcacacgagggggctggacttcgcctgtgatatctacatctgggcgcccttggccgggacttgtggggtccttctcctgtcactggttatcaccctttactgcaaacggggcagaaagaaactcctgtatatattcaaacaaccatttatgagaccagtacaaactactcaagaggaagatggctgtagctgccgatttccagaagaagaagaaggaggatgtgaactgagagtgaagttcagcaggagcgcagacgcccccgcgtaccagcagggccagaaccagctctataacgagctcaatctaggacgaagagaggagtacgatgttttggacaagagacgtggccgggaccctgagatggggggaaagccgagaaggaagaaccctcaggaaggcctgtacaatgaactgcagaaagataagatggcggaggcctacagtgagattgggatgaaaggcgagcgccggaggggcaaggggcacgatggcctttaccagggtctcagtacagccaccaaggacacctacgacgcccttcacatgcaggccctgccccctcgctaa

SEQ ID NO: 36 - DNA, 1473 bp, synthetic construct
  source 1..1473: mol_type = other DNA
atggccttaccagtgaccgccttgctcctgccgctggccttgctgctccacgccgccaggccggagatcgtgatgacccagtccccaagtacactgagcgcctccgtgggcgaccgcgtgatcataaactgtcaggcctcccagtctatcgacagctggttgtcatggtatcaacagaagcccggtaaggcccccaaactgctcatttacctggcatccacactggcatccggggtgccaagccgcttctccgggagtgggtctggcgccgagttcaccctgaccatatcttccctgcagcccgacgacttcgcaacgtactattgccaaagtaacgatgagagtagcatctacggtgccgccttcgggcagggcacgaagttgaccgtgctgggcggagggggctcaggaggtggcggtagcggaggaggcggctcagaagtgcagctggtggagtccggcggtggactggtgcaaccgggaggctcactcagattgtcatgcaccgcctctggctttagtctttcaatttacgacatgatatgggtgaggcaggcacccggcaagggcctggaatggatcggcattattatttacgggggcagtgccagctacgcgaattgggcgaagggcaggtttaccatcagccgcgacaacagcaagaataccgtttacctgcagatgaatagcctgagggccgaagacacggcggtctatttctgtgcacggggtgcatcatcatacagttactcttatggcttctccctgtggggccctgggaccctcgtaactgtgagcagcaccacgacgccagcgccgcgaccaccaacaccggcgcccaccatcgcgtcgcagcccctgtccctgcgcccagaggcgtgccggccagcggcggggggcgcagtgcacacgagggggctggacttcgcctgtgatatctacatctgggcgcccttggccgggacttgtggggtccttctcctgtcactggttatcaccctttactgcaaacggggcagaaagaaactcctgtatatattcaaacaaccatttatgagaccagtacaaactactcaagaggaagatggctgtagctgccgatttccagaagaagaagaaggaggatgtgaactgagagtgaagttcagcaggagcgcagacgcccccgcgtaccagcagggccagaaccagctctataacgagctcaatctaggacgaagagaggagtacgatgttttggacaagagacgtggccgggaccctgagatggggggaaagccgagaaggaagaaccctcaggaaggcctgtacaatgaactgcagaaagataagatggcggaggcctacagtgagattgggatgaaaggcgagcgccggaggggcaaggggcacgatggcctttaccagggtctcagtacagccaccaaggacacctacgacgcccttcacatgcaggccctgccccctcgctaa

SEQ ID NO: 37 - protein, 15 aa, synthetic construct
GGGGSGGGGSGGGGS

SEQ ID NO: 38 - protein, 18 aa, synthetic construct
GSTSGSGKPGSGEGSTKG

SEQ ID NO: 39 - protein, 18 aa, synthetic construct
GSTSGGGSGGGSGGGGSS

SEQ ID NO: 40 - protein, 246 aa, synthetic construct
DIVLTQSPPSLAMSLGKRATISCRASESVTILGSHLIHWYQQKPGQPPTLLIQLASNVQTGVPARFSGSGSRTDFTLTIDPVEEDDVAVYYCLQSRTIPRTFGGGTKLEIKGSTSGSGKPGSGEGSTKGQIQLVQSGPELKKPGETVKISCKASGYTFTDYSINWVKRAPGKGLKWMGWINTETREPAYAYDFRGRFAFSLETSASTAYLQINNLKYEDTATYFCALDYSYAMDYWGQGTSVTVSS

SEQ ID NO: 41 - DNA, 738 bp, synthetic construct
  source 1..738: mol_type = other DNA
gacattgtgctcactcagtcacctcccagcctggccatgagcctgggaaaaagggccaccatctcctgtagagccagtgagtccgtcacaatcttggggagccatcttattcactggtatcagcagaagcccgggcagcctccaacccttcttattcagctcgcgtcaaacgtccagacgggtgtacctgccagattttctggtagcgggtcccgcactgattttacactgaccatagatccagtggaagaagacgatgtggccgtgtattattgtctgcagagcagaacgattcctcgcacatttggtgggggtactaagctggagattaagggaagcacgtccggctcagggaagccgggctccggcgagggaagcacgaaggggcaaattcagctggtccagagcggacctgagctgaaaaaacccggcgagactgttaagatcagttgtaaagcatctggctataccttcaccgactacagcataaattgggtgaaacgggcccctggaaagggcctcaaatggatgggttggatcaataccgaaactagggagcctgcttatgcatatgacttccgcgggagattcgccttttcactcgagacatctgcctctactgcttacctccaaataaacaacctcaagtatgaagatacagccacttacttttgcgccctcgactatagttacgccatggactactggggacagggaacctccgttaccgtcagttcc